European Patent Specification EP 3 795 592 B1, published July 24, 2024. Title: OPTIMIZATION OF ANTIBODIES THAT BIND LYMPHOCYTE ACTIVATION GENE-3 (LAG-3), AND USES THEREOF. Applicant: Bristol-Myers Squibb Company. The sequence listing filed with the application follows.

SEQUENCE LISTING (52 sequences)

SEQ ID NO: 1 - DNA, 360 bp, Artificial Sequence
  source: /note="Description of Artificial Sequence: Synthetic polynucleotide"
  CDS (1)..(360)
caggtgcagctacagcagtggggcgcaggactgttgaagccttcggagaccctgtccctcacctgcgctgtctatggtgggtccttcagtgattactactggaactggatccgccagcccccagggaaggggctggagtggattggggaaatcaatcataatggaaacaccaactccaacccgtccctcaagagtcgagtcaccctatcactagacacgtccaagaaccagttctccctgaagctgaggtctgtgaccgccgcggacacggctgtgtattactgtgcgtttggatatagtgactacgagtacaactggttcgacccctggggccagggaaccctggtcaccgtctcctca

SEQ ID NO: 2 - protein, 120 aa, Artificial Sequence
  source: /note="Description of Artificial Sequence: Synthetic polypeptide"
QVQLQQWGAGLLKPSETLSLTCAVYGGSFSDYYWNWIRQPPGKGLEWIGEINHNGNTNSNPSLKSRVTLSLDTSKNQFSLKLRSVTAADTAVYYCAFGYSDYEYNWFDPWGQGTLVTVSS

SEQ ID NO: 3 - DNA, 321 bp, Artificial Sequence
  source: /note="Description of Artificial Sequence: Synthetic polynucleotide"
  CDS (1)..(321)
gaaattgtgttgacacagtctccagccaccctgtctttgtctccaggggaaagagccaccctctcctgcagggccagtcagagtattagcagctacttagcctggtaccaacagaaacctggccaggctcccaggctcctcatctatgatgcatccaacagggccactggcatcccagccaggttcagtggcagtgggtctgggacagacttcactctcaccatcagcagcctagagcctgaagattttgcagtttattactgtcagcagcgtagcaactggcctctcacttttggccaggggaccaacctggagatcaaa

SEQ ID NO: 4 - protein, 107 aa, Artificial Sequence
  source: /note="Description of Artificial Sequence: Synthetic polypeptide"
EIVLTQSPATLSLSPGERATLSCRASQSISSYLAWYQQKPGQAPRLLIYDASNRATGIPARFSGSGSGTDFTLTISSLEPEDFAVYYCQQRSNWPLTFGQGTNLEIK

SEQ ID NO: 5 - protein, 5 aa, Artificial Sequence
  source: /note="Description of Artificial Sequence: Synthetic peptide"
DYYWN

SEQ ID NO: 6 - protein, 16 aa, Artificial Sequence
  source: /note="Description of Artificial Sequence: Synthetic peptide"
EINHNGNTNSNPSLKS

SEQ ID NO: 7 - protein, 12 aa, Artificial Sequence
  source: /note="Description of Artificial Sequence: Synthetic peptide"
GYSDYEYNWFDP

SEQ ID NO: 8 - protein, 11 aa, Artificial Sequence
  source: /note="Description of Artificial Sequence: Synthetic peptide"
RASQSISSYLA

SEQ ID NO: 9 - protein, 7 aa, Artificial Sequence
  source: /note="Description of Artificial Sequence: Synthetic peptide"
DASNRAT

SEQ ID NO: 10 - protein, 9 aa, Artificial Sequence
  source: /note="Description of Artificial Sequence: Synthetic peptide"
QQRSNWPLT

SEQ ID NO: 11 - DNA, 360 bp, Artificial Sequence
  source: /note="Description of Artificial Sequence: Synthetic polynucleotide"
caggtgcagctacagcagtggggcgcaggactgttgaagccttcggagaccctgtccctcacctgcgctgtctatggtgggtccttcagtgattactactggaactggatccgccagcccccagggaaggggctggagtggattggggaaatcaatcatcgtggaagcaccaactccaacccgtccctcaagagtcgagtcaccctatcactagacacgtccaagaaccagttctccctgaagctgaggtctgtgaccgccgcggacacggctgtgtattactgtgcgtttggatatagtgactacgagtacaactggttcgacccctggggccagggaaccctggtcaccgtctcctca

SEQ ID NO: 12 - protein, 120 aa, Artificial Sequence
  source: /note="Description of Artificial Sequence: Synthetic polypeptide"
QVQLQQWGAGLLKPSETLSLTCAVYGGSFSDYYWNWIRQPPGKGLEWIGEINHRGSTNSNPSLKSRVTLSLDTSKNQFSLKLRSVTAADTAVYYCAFGYSDYEYNWFDPWGQGTLVTVSS

SEQ ID NO: 13 - DNA, 321 bp, Artificial Sequence; identical to SEQ ID NO: 3
  source: /note="Description of Artificial Sequence: Synthetic polynucleotide"
  CDS (1)..(321)

SEQ ID NO: 14 - protein, 107 aa, Artificial Sequence; identical to SEQ ID NO: 4
  source: /note="Description of Artificial Sequence: Synthetic polypeptide"

SEQ ID NO: 15 - protein, 5 aa, Artificial Sequence
  source: /note="Description of Artificial Sequence: Synthetic peptide"
DYYWN

SEQ ID NO: 16 - protein, 16 aa, Artificial Sequence
  source: /note="Description of Artificial Sequence: Synthetic peptide"
EINHRGSTNSNPSLKS

SEQ ID NO: 17 - protein, 12 aa, Artificial Sequence
  source: /note="Description of Artificial Sequence: Synthetic peptide"
GYSDYEYNWFDP

SEQ ID NO: 18 - protein, 11 aa, Artificial Sequence
  source: /note="Description of Artificial Sequence: Synthetic peptide"
RASQSISSYLA

SEQ ID NO: 19 - protein, 7 aa, Artificial Sequence
  source: /note="Description of Artificial Sequence: Synthetic peptide"
DASNRAT

SEQ ID NO: 20 - protein, 9 aa, Artificial Sequence
  source: /note="Description of Artificial Sequence: Synthetic peptide"
QQRSNWPLT

SEQ ID NO: 21 - protein, 8 aa, Homo sapiens
PGHPLAPG

SEQ ID NO: 22 - protein, 8 aa, Homo sapiens
HPAAPSSW

SEQ ID NO: 23 - protein, 8 aa, Homo sapiens
PAAPSSWG

SEQ ID NO: 24 - protein, 16 aa, Artificial Sequence
  source: /note="Description of Artificial Sequence: Synthetic peptide"
EIIHSGSTNSNPSLKS

SEQ ID NO: 25 - protein, 16 aa, Artificial Sequence
  source: /note="Description of Artificial Sequence: Synthetic peptide"
EINHGGGTNSNPSLKS

SEQ ID NO: 26 - protein, 16 aa, Artificial Sequence
  source: /note="Description of Artificial Sequence: Synthetic peptide"
EINHIGNTNSNPSLKS

SEQ ID NO: 27 - protein, 11 aa, Homo sapiens
GEINHSGSTNY

SEQ ID NO: 28 - protein, 15 aa, Artificial Sequence
  source: /note="Description of Artificial Sequence: Synthetic peptide"
GGGGSGGGGSGGGGS

SEQ ID NO: 29 - protein, 525 aa, Homo sapiens
MWEAQFLGLLFLQPLWVAPVKPLQPGAEVPVVWAQEGAPAQLPCSPTIPLQDLSLLRRAGVTWQHQPDSGPPAAAPGHPLAPGPHPAAPSSWGPRPRRYTVLSVGPGGLRSGRLPLQPRVQLDERGRQRGDFSLWLRPARRADAGEYRAAVHLRDRALSCRLRLRLGQASMTASPPGSLRASDWVILNCSFSRPDRPASVHWFRNRGQGRVPVRESPHHHLAESFLFLPQVSPMDSGPWGCILTYRDGFNVSIMYNLTVLGLEPPTPLTVYAGAGSRVGLPCRLPAGVGTRSFLTAKWTPPGGGPDLLVTGDNGDFTLRLEDVSQAQAGTYTCHIHLQEQQLNATVTLAIITVTPKSFGSPGSLGKLLCEVTPVSGQERFVWSSLDTPSQRSFSGPWLEAQEAQLLSQPWQCQLYQGERLLGAAVYFTELSSPGAQRSGRAPGALPAGHLLLFLTLGVLSLLLLVTGAFGFHLWRRQWRPRRFSALEQGIHPPQAQSKIEELEQEPEPEPEPEPEPEPEPEPEQL

SEQ ID NO: 30 - protein, 17 aa, Artificial Sequence
  source: /note="Description of Artificial Sequence: Synthetic peptide"
VIWYDGSNKYYADSVKG

SEQ ID NO: 31 - DNA, 1344 bp, Artificial Sequence
  source: /note="Description of Artificial Sequence: Synthetic polynucleotide"
caggtgcagctacagcagtggggcgcaggactgttgaagccttcggagaccctgtccctcacctgcgctgtctatggtgggtccttcagtgattactactggaactggatccgccagcccccagggaaggggctggagtggattggggaaatcaatcataatggaaacaccaactccaacccgtccctcaagagtcgagtcaccctatcactagacacgtccaagaaccagttctccctgaagctgaggtctgtgaccgccgcggacacggctgtgtattactgtgcgtttggatatagtgactacgagtacaactggttcgacccctggggccagggaaccctggtcaccgtctcctcagctagcaccaagggcccatccgtcttccccctggcgccctgctccaggagcacctccgagagcacagccgccctgggctgcctggtcaaggactacttccccgaaccggtgacggtgtcgtggaactcaggcgccctgaccagcggcgtgcacaccttcccggctgtcctacagtcctcaggactctactccctcagcagcgtggtgaccgtgccctccagcagcttgggcacgaagacctacacctgcaacgtagatcacaagcccagcaacaccaaggtggacaagagagttgagtccaaatatggtcccccatgcccaccatgcccagcacctgagttcctggggggaccatcagtcttcctgttccccccaaaacccaaggacactctcatgatctcccggacccctgaggtcacgtgcgtggtggtggacgtgagccaggaagaccccgaggtccagttcaactggtacgtggatggcgtggaggtgcataatgccaagacaaagccgcgggaggagcagttcaacagcacgtaccgtgtggtcagcgtcctcaccgtcctgcaccaggactggctgaacggcaaggagtacaagtgcaaggtctccaacaaaggcctcccgtcctccatcgagaaaaccatctccaaagccaaagggcagccccgagagccacaggtgtacaccctgcccccatcccaggaggagatgaccaagaaccaggtcagcctgacctgcctggtcaaaggcttctaccccagcgacatcgccgtggagtgggagagcaatgggcagccggagaacaactacaagaccacgcctcccgtgctggactccgacggctccttcttcctctacagcaggctaaccgtggacaagagcaggtggcaggaggggaatgtcttctcatgctccgtgatgcatgaggctctgcacaaccactacacacagaagagcctctccctgtctctgggtaaatga

SEQ ID NO: 32 - protein, 447 aa, Artificial Sequence
  source: /note="Description of Artificial Sequence: Synthetic polypeptide"
QVQLQQWGAGLLKPSETLSLTCAVYGGSFSDYYWNWIRQPPGKGLEWIGEINHNGNTNSNPSLKSRVTLSLDTSKNQFSLKLRSVTAADTAVYYCAFGYSDYEYNWFDPWGQGTLVTVSSASTKGPSVFPLAPCSRSTSESTAALGCLVKDYFPEPVTVSWNSGALTSGVHTFPAVLQSSGLYSLSSVVTVPSSSLGTKTYTCNVDHKPSNTKVDKRVESKYGPPCPPCPAPEFLGGPSVFLFPPKPKDTLMISRTPEVTCVVVDVSQEDPEVQFNWYVDGVEVHNAKTKPREEQFNSTYRVVSVLTVLHQDWLNGKEYKCKVSNKGLPSSIEKTISKAKGQPREPQVYTLPPSQEEMTKNQVSLTCLVKGFYPSDIAVEWESNGQPENNYKTTPPVLDSDGSFFLYSRLTVDKSRWQEGNVFSCSVMHEALHNHYTQKSLSLSLGK

SEQ ID NO: 33 - DNA, 645 bp, Artificial Sequence
  source: /note="Description of Artificial Sequence: Synthetic polynucleotide"
gaaattgtgttgacacagtctccagccaccctgtctttgtctccaggggaaagagccaccctctcctgcagggccagtcagagtattagcagctacttagcctggtaccaacagaaacctggccaggctcccaggctcctcatctatgatgcatccaacagggccactggcatcccagccaggttcagtggcagtgggtctgggacagacttcactctcaccatcagcagcctagagcctgaagattttgcagtttattactgtcagcagcgtagcaactggcctctcacttttggccaggggaccaacctggagatcaaacgtacggtggctgcaccatctgtcttcatcttcccgccatctgatgagcagttgaaatctggaactgcctctgttgtgtgcctgctgaataacttctatcccagagaggccaaagtacagtggaaggtggataacgccctccaatcgggtaactcccaggagagtgtcacagagcaggacagcaaggacagcacctacagcctcagcagcaccctgacgctgagcaaagcagactacgagaaacacaaagtctacgcctgcgaagtcacccatcagggcctgagctcgcccgtcacaaagagcttcaacaggggagagtgttag

SEQ ID NO: 34 - protein, 214 aa, Artificial Sequence
  source: /note="Description of Artificial Sequence: Synthetic polypeptide"
EIVLTQSPATLSLSPGERATLSCRASQSISSYLAWYQQKPGQAPRLLIYDASNRATGIPARFSGSGSGTDFTLTISSLEPEDFAVYYCQQRSNWPLTFGQGTNLEIKRTVAAPSVFIFPPSDEQLKSGTASVVCLLNNFYPREAKVQWKVDNALQSGNSQESVTEQDSKDSTYSLSSTLTLSKADYEKHKVYACEVTHQGLSSPVTKSFNRGEC

SEQ ID NO: 35 - protein, 447 aa, Artificial Sequence
  source: /note="Description of Artificial Sequence: Synthetic polypeptide"
QVQLQQWGAGLLKPSETLSLTCAVYGGSFSDYYWNWIRQPPGKGLEWIGEINHRGSTNSNPSLKSRVTLSLDTSKNQFSLKLRSVTAADTAVYYCAFGYSDYEYNWFDPWGQGTLVTVSSASTKGPSVFPLAPCSRSTSESTAALGCLVKDYFPEPVTVSWNSGALTSGVHTFPAVLQSSGLYSLSSVVTVPSSSLGTKTYTCNVDHKPSNTKVDKRVESKYGPPCPPCPAPEFLGGPSVFLFPPKPKDTLMISRTPEVTCVVVDVSQEDPEVQFNWYVDGVEVHNAKTKPREEQFNSTYRVVSVLTVLHQDWLNGKEYKCKVSNKGLPSSIEKTISKAKGQPREPQVYTLPPSQEEMTKNQVSLTCLVKGFYPSDIAVEWESNGQPENNYKTTPPVLDSDGSFFLYSRLTVDKSRWQEGNVFSCSVMHEALHNHYTQKSLSLSLGK

SEQ ID NO: 36 - DNA, 1344 bp, Artificial Sequence
  source: /note="Description of Artificial Sequence: Synthetic polynucleotide"
caggtgcagctacagcagtggggcgcaggactgttgaagccttcggagaccctgtccctcacctgcgctgtctatggtgggtccttcagtgattactactggaactggatccgccagcccccagggaaggggctggagtggattggggaaatcaatcatcgtggaagcaccaactccaacccgtccctcaagagtcgagtcaccctatcactagacacgtccaagaaccagttctccctgaagctgaggtctgtgaccgccgcggacacggctgtgtattactgtgcgtttggatatagtgactacgagtacaactggttcgacccctggggccagggaaccctggtcaccgtctcctcagctagcaccaagggcccatccgtcttccccctggcgccctgctccaggagcacctccgagagcacagccgccctgggctgcctggtcaaggactacttccccgaaccggtgacggtgtcgtggaactcaggcgccctgaccagcggcgtgcacaccttcccggctgtcctacagtcctcaggactctactccctcagcagcgtggtgaccgtgccctccagcagcttgggcacgaagacctacacctgcaacgtagatcacaagcccagcaacaccaaggtggacaagagagttgagtccaaatatggtcccccatgcccaccatgcccagcacctgagttcctggggggaccatcagtcttcctgttccccccaaaacccaaggacactctcatgatctcccggacccctgaggtcacgtgcgtggtggtggacgtgagccaggaagaccccgaggtccagttcaactggtacgtggatggcgtggaggtgcataatgccaagacaaagccgcgggaggagcagttcaacagcacgtaccgtgtggtcagcgtcctcaccgtcctgcaccaggactggctgaacggcaaggagtacaagtgcaaggtctccaacaaaggcctcccgtcctccatcgagaaaaccatctccaaagccaaagggcagccccgagagccacaggtgtacaccctgcccccatcccaggaggagatgaccaagaaccaggtcagcctgacctgcctggtcaaaggcttctaccccagcgacatcgccgtggagtgggagagcaatgggcagccggagaacaactacaagaccacgcctcccgtgctggactccgacggctccttcttcctctacagcaggctaaccgtggacaagagcaggtggcaggaggggaatgtcttctcatgctccgtgatgcatgaggctctgcacaaccactacacacagaagagcctctccctgtctctgggtaaatga

SEQ ID NO: 37 - protein, 214 aa, Artificial Sequence; identical to SEQ ID NO: 34
  source: /note="Description of Artificial Sequence: Synthetic polypeptide"

SEQ ID NO: 38 - DNA, 645 bp, Artificial Sequence; identical to SEQ ID NO: 33
  source: /note="Description of Artificial Sequence: Synthetic polynucleotide"

SEQ ID NO: 39 - protein, 5 aa, Artificial Sequence
  source: /note="Description of Artificial Sequence: Synthetic peptide"
PVGVV

SEQ ID NO: 40 - protein, 13 aa, Artificial Sequence
  source: /note="Description of Artificial Sequence: Synthetic peptide"
GEINHRGSTNSNP

SEQ ID NO: 41 - protein, 11 aa, Artificial Sequence
  source: /note="Description of Artificial Sequence: Synthetic peptide"
GEINHNGNTNS

SEQ ID NO: 42 - protein, 11 aa, Artificial Sequence
  source: /note="Description of Artificial Sequence: Synthetic peptide"
GEINHRGSTNS

SEQ ID NO: 43 - protein, 11 aa, Artificial Sequence
  source: /note="Description of Artificial Sequence: Synthetic peptide"
GEIIHSGSTNS

SEQ ID NO: 44 - protein, 11 aa, Artificial Sequence
  source: /note="Description of Artificial Sequence: Synthetic peptide"
GEINHGGGTNS

SEQ ID NO: 45 - protein, 11 aa, Artificial Sequence
  source: /note="Description of Artificial Sequence: Synthetic peptide"
GEINHIGNTNS

SEQ ID NO: 46 - protein, 14 aa, Artificial Sequence
  source: /note="Description of Artificial Sequence: Synthetic peptide"
  MOD_RES (4)..(4): Isomerized residue
INHDGNTNSNPSLK

SEQ ID NO: 47 - protein, 14 aa, Artificial Sequence
  source: /note="Description of Artificial Sequence: Synthetic peptide"
INHDGNTNSNPSLK

SEQ ID NO: 48 - protein, 14 aa, Artificial Sequence
  source: /note="Description of Artificial Sequence: Synthetic peptide"
INHNGNTDSNPSLK

SEQ ID NO: 49 - protein, 14 aa, Artificial Sequence
  source: /note="Description of Artificial Sequence: Synthetic peptide"
IDHNGNTNSNPSLK

SEQ ID NO: 50 - protein, 14 aa, Artificial Sequence
  source: /note="Description of Artificial Sequence: Synthetic peptide"
  MOD_RES (8)..(8): Isomerized residue
INHRGSTDSNPSLK

SEQ ID NO: 51 - protein, 14 aa, Artificial Sequence
  source: /note="Description of Artificial Sequence: Synthetic peptide"
INHRGSTNSNPSLK

SEQ ID NO: 52 - protein, 14 aa, Artificial Sequence
  source: /note="Description of Artificial Sequence: Synthetic peptide"
  MOD_RES (2)..(2): Isomerized residue
IDHRGSTDSNPSLK